European Patent Specification EP 4 143 346 B1, published January 7, 2026. Title: METHOD FOR EARLY DETECTION, PREDICTION OF TREATMENT RESPONSE AND PROGNOSIS OF COLORECTAL CANCER. Applicant: TAIPEI MEDICAL UNIVERSITY. Application 63/017,309. The sequence listing filed with the application follows.

SEQUENCE LISTING (16 sequences)

SEQ ID NO: 1 - DNA, 27 bp, Artificial Sequence
  primer
tttagaattatgaagattatggtgttc

SEQ ID NO: 2 - DNA, 20 bp, Artificial Sequence
  primer
aaaactcaacatcgaaccga

SEQ ID NO: 3 - DNA, 22 bp, Artificial Sequence
  primer
cgaccccgcccgatatccataa

SEQ ID NO: 4 - DNA, 27 bp, Artificial Sequence
  probe
tttagaattatgaagattatggtgttc

SEQ ID NO: 5 - DNA, 25 bp, Artificial Sequence
  primer
ggtgagtttttgatttgtaattgtc

SEQ ID NO: 6 - DNA, 23 bp, Artificial Sequence
  primer
atctcgtaccgctactactacgc

SEQ ID NO: 7 - DNA, 28 bp, Artificial Sequence
  probe
gtcgggggttgttgattttagtagcgtt

SEQ ID NO: 8 - DNA, 19 bp, Artificial Sequence
  primer
gtttgggttttggggagtc

SEQ ID NO: 9 - DNA, 19 bp, Artificial Sequence
  primer
gatcgaacaactcaacccg

SEQ ID NO: 10 - DNA, 20 bp, Artificial Sequence
  primer
gtttttgtgcggtttttgga

SEQ ID NO: 11 - DNA, 20 bp, Artificial Sequence
  primer
aaccgcgaacgaaaactaaa

SEQ ID NO: 12 - DNA, 20 bp, Artificial Sequence
  probe
cgaaaataaaaatccgacga

SEQ ID NO: 13 - DNA, 20 bp, Artificial Sequence
  probe
ttgttacgcgttgttcgtgt

SEQ ID NO: 14 - DNA, 25 bp, Artificial Sequence
  primer
gaataaggtcgttagttattatcgt

SEQ ID NO: 15 - DNA, 22 bp, Artificial Sequence
  primer
aatcaaatctacccgaatcgaa

SEQ ID NO: 16 - DNA, 36 bp, Artificial Sequence
  probe
gaaagaaagaaagaaagtaaattttatttttaagcg